European Patent Specification EP 3 432 923 B1, published August 2, 2023. Title: HCV VACCINES. Applicant: OXFORD UNIVERSITY INNOVATION LIMITED. Application EP 17715523.1. The sequence listing filed with the application follows.

SEQUENCE LISTING (195 sequences)

SEQ ID NO: 1 - protein, 191 aa, Homo sapiens
MSTNPKPQRKTKRNTNRRPQDVKFPGGGQIVGGVYLLPRRGPRLGVRATRKTSERSQPRGRRQPIPKARRPEGRTWAQPGYPWPLYGNEGCGWAGWLLSPRGSRPSWGPTDPRRRSRNLGKVIDTLTCGFADLMGYIPLVGAPLGGAARALAHGVRVLEDGVNYATGNLPGCSFSIFLLALLSCLTVPASA

SEQ ID NO: 2 - protein, 21 aa, Homo sapiens
YVGDLCGSVFLVSQLFTFSPR

SEQ ID NO: 3 - protein, 20 aa, Homo sapiens
YPGHITGHRMAWDMMMNWSP

SEQ ID NO: 4 - protein, 20 aa, Homo sapiens
VCGPVYCFTPSPVVVGTTDR

SEQ ID NO: 5 - protein, 22 aa, Homo sapiens
TDVFLLNNTRPPLGNWFGCTWM

SEQ ID NO: 6 - protein, 36 aa, Homo sapiens
CPTDCFRKHPEATYSRCGSGPWLTPRCLVDYPYRLW

SEQ ID NO: 7 - protein, 54 aa, Homo sapiens
DRDRSELSPLLLSTTEWQVLPCSFTTLPALSTGLIHLHQNIVDVQYLYGVGSSV

SEQ ID NO: 8 - protein, 54 aa, Homo sapiens
DRDRSELSPLLLSTTQWQVLPCSFTTLPALSTGLIHLHQNIVDVQYLYGVGSSV

SEQ ID NO: 9 - protein, 24 aa, Homo sapiens
ARVCACLWMMLLIAQAEAALENLV

SEQ ID NO: 10 - protein, 44 aa, Homo sapiens
QGWRLLAPITAYAQQTRGLLGCIITSLTGRDKNQVEGEVQIVST

SEQ ID NO: 11 - protein, 44 aa, Homo sapiens
KGWRLLAPITAYAQQTRGLLGCIITSLTGRDKNQVEGEVQIVST

SEQ ID NO: 12 - protein, 20 aa, Homo sapiens
QSFLATCINGVCWTVYHGAG

SEQ ID NO: 13 - protein, 153 aa, Homo sapiens
PCTCGSSDLYLVTRHADVIPVRRRGDSRGSLLSPRPISYLKGSSGGPLLCPSGHAVGIFRAAVCTRGVAKAVDFIPVESLETTMRSPVFTDNSSPPAVPQTFQVAHLHAPTGSGKSTKVPAAYAAQGYKVLVLNPSVAATLGFGAYMSKAHGV

SEQ ID NO: 14 - protein, 153 aa, Homo sapiens
PCTCGSSDLYLVTRHADVIPVRRRGDSRGSLLSPRPISYLKGSSGGPLLCPSGHAVGIFRAAVCTRGVAKAVDFIPVESMETTMRSPVFTDNSSPPAVPQTFQVAHLHAPTGSGKSTKVPAAYAAQGYKVLVLNPSVAATLGFGAYMSKAHGV

SEQ ID NO: 15 - protein, 86 aa, Homo sapiens
TGVRTITTGAPITYSTYGKFLADGGCSGGAYDIIICDECHSTDATSILGIGTVLDQAETAGARLVVLATATPPGSVTVPHPNIEEV

SEQ ID NO: 16 - protein, 86 aa, Homo sapiens
TGVRTITTGSPITYSTYGKFLADGGCSGGAYDIIICDECHSTDATSILGIGTVLDQAETAGARLVVLATATPPGSVTVPHPNIEEV

SEQ ID NO: 17 - protein, 83 aa, Homo sapiens
NAVAYYRGLDVSVIPTSGDVVVVATDALMTGFTGDFDSVIDCNTCVTQTVDFSLDPTFTIETTTLPQDAVSRTQRRGRTGRGR

SEQ ID NO: 18 - protein, 118 aa, Homo sapiens
YRFVTPGERPSGMFDSSVLCECYDAGCAWYELTPAETTVRLRAYLNTPGLPVCQDHLEFWEGVFTGLTHIDAHFLSQTKQAGENFPYLVAYQATVCARAQAPPPSWDQMWKCLIRLKP

SEQ ID NO: 19 - protein, 118 aa, Homo sapiens
YRFVTPGERPSGMFDSSVLCECYDAGCAWYELTPAETTVRLRAYLNTPGLPVCQDHLEFWEGVFTGLTHIDAHFLSQTKQAGDNFPYLVAYQATVCARAQAPPPSWDQMWKCLIRLKP

SEQ ID NO: 20 - protein, 48 aa, Homo sapiens
KYIMTCMSADLEVVTSTWVLVGGVLAALAAYCLSTGCVVIVGRIVLSG

SEQ ID NO: 21 - protein, 45 aa, Homo sapiens
FWAKHMWNFISGIQYLAGLSTLPGNPAIASLMAFTAAVTSPLTTQ

SEQ ID NO: 22 - protein, 45 aa, Homo sapiens
FWAKHMWNFISGIQYLAGLSTLPGNPAIASLMAFTASVTSPLTTQ

SEQ ID NO: 23 - protein, 110 aa, Homo sapiens
GSIGLGKVLVDILAGYGAGVAGALVAFKIMSGEVPSTEDLVNLLPAILSPGALVVGVVCAAILRRHVGPGEGAVQWMNRLIAFASRGNHVSPTHYVPESDAAARVTQILS

SEQ ID NO: 24 - protein, 22 aa, Homo sapiens
SWLRDIWDWICEVLSDFKTWLK

SEQ ID NO: 25 - protein, 21 aa, Homo sapiens
CPCQVPSPEFFTELDGVRLHR

SEQ ID NO: 26 - protein, 32 aa, Homo sapiens
RRLARGSPPSLASSSASQLSAPSLKATCTTNH

SEQ ID NO: 27 - protein, 33 aa, Homo sapiens
SDAESYSSMPPLEGEPGDPDLSDGSWSTVSSEE

SEQ ID NO: 28 - protein, 33 aa, Homo sapiens
SDAESYSSMPPLEGEPGDPDLSDGSWSTVSSEA

SEQ ID NO: 29 - protein, 20 aa, Homo sapiens
LSNSLLRHHNMVYATTSRSA

SEQ ID NO: 30 - protein, 21 aa, Homo sapiens
LTPPHSAKSKFGYGAKDVRCH

SEQ ID NO: 31 - protein, 25 aa, Homo sapiens
KPARLIVFPDLGVRVCEKMALYDVV

SEQ ID NO: 32 - protein, 23 aa, Homo sapiens
PMGFSYDTRCFDSTVTESDIRTE

SEQ ID NO: 33 - protein, 54 aa, Homo sapiens
SLTERLYVGGPLTNSKGQNCGYRRCRASGVLTTSCGNTLTCYLKASAACRAAKL

SEQ ID NO: 34 - protein, 23 aa, Homo sapiens
CTMLVCGDDLVVICESAGTQEDA

SEQ ID NO: 35 - protein, 91 aa, Homo sapiens
SLRAFTEAMTRYSAPPGDPPQPEYDLELITSCSSNVSVAHDASGKRVYYLTRDPTTPLARAAWETARHTPVNSWLGNIIMFAPTLWARMIL

SEQ ID NO: 36 - protein, 91 aa, Homo sapiens
SLRAFTEAMTRYSAPPGDPPQPEYDLELITSCSSNVSVAHDASGKRVYYLTRDPTTPLARAAWETARHTPVNSWLGNIIMYAPTLWARMIL

SEQ ID NO: 37 - protein, 55 aa, Homo sapiens
EPLDLPQIIQRLHGLSAFSLHSYSPGEINRVAACLRKLGVPPLRAWRHRARSVRA

SEQ ID NO: 38 - protein, 28 aa, Homo sapiens
GGRAAICGKYLFNWAVRTKLKLTPIPAA

SEQ ID NO: 39 - protein, 190 aa, Homo sapiens
MSTLPKPQRKTKRNTNRRPQDVKFPGGGQIVGGVYLLPRRGPRLGVRATRKTSERSQPRGRRQPIPKARRPEGRSWAQPGYPWPLYGNEGCGWAGWLLSPRGSRPSWGPNDPRRRSRNLGKVIDTLTCGFADLMGYIPLVGAPLGGVARALAHGVRALEDGVNFATGNLPGCSFSIFLLALLSCLTHPAS

SEQ ID NO: 40 - protein, 190 aa, Homo sapiens
MSTNPKPQRKTKRNTNRRPQDVKFPGGGQIVGGVYLLPRRGPRLGVRATRKTSERSQPRGRRQPIPKARRPEGRSWAQPGYPWPLYGNEGCGWAGWLLSPRGSRPSWGPTDPRRRSRNLGKVIDTLTCGFADLMGYIPLVGAPLGGAARALAHGVRVLEDGVNYATGNLPGCSFSIFLLALLSCLTVPAS

SEQ ID NO: 41 - protein, 21 aa, Homo sapiens
VDLLVGAATMCSALYVGDLCG

SEQ ID NO: 42 - protein, 21 aa, Homo sapiens
VDLLVGAATMCSALYVGDLCG

SEQ ID NO: 43 - protein, 20 aa, Homo sapiens
HWGVLAGLAYYSMQGNWAKV

SEQ ID NO: 44 - protein, 21 aa, Homo sapiens
SVCGPVYCFTPSPVVVGTTDR

SEQ ID NO: 45 - protein, 26 aa, Homo sapiens
RCGSGPWLTPRCLVDYPYRLWHYPCT

SEQ ID NO: 46 - protein, 21 aa, Homo sapiens
AACNWTRGERCDIEDRDRSEL

SEQ ID NO: 47 - protein, 41 aa, Homo sapiens
TTELAILPCSFTPLPALSTGLIHLHQNIVDVQYLYGVGSGM

SEQ ID NO: 48 - protein, 45 aa, Homo sapiens
MGWRLLAPITAYAQQTRGLLGCIVTSLTGRDKNVVEGEVQVLSTA

SEQ ID NO: 49 - protein, 45 aa, Homo sapiens
MGWRLLAPITAYAQQTRGLLGTIVTSLTGRDKNVVTGEVQVLSTA

SEQ ID NO: 50 - protein, 80 aa, Homo sapiens
PCTCGSSDLYLVTRHADVIPARRRGDSRASLLSPRPLAYLKGSSGGPLLCPSGHVAGIFRAAVCTRGVAKALQFIPVETL

SEQ ID NO: 51 - protein, 80 aa, Homo sapiens
PCTCGSADLYLVTRDADVIPARRRGDSTASLLSPRPLACLKGSSGGPVMCPSGHVAGIFRAAVCTRGVAKALQFIPVETL

SEQ ID NO: 52 - protein, 66 aa, Homo sapiens
RSPSFSDNSTPPAVPQSYQVAHLHAPTGSGKSTKVPAAYAAQGYKVLVLNPSVAATLGFGAYMSKA

SEQ ID NO: 53 - protein, 66 aa, Homo sapiens
RSPVFSDNSSPPAVPQSYQVAHLHAPTGSGKSTKVPAAYAAQGYKVLVLNPSVAATLGFGAYMSKA

SEQ ID NO: 54 - protein, 88 aa, Homo sapiens
TGNRTITTGAKITYSTYGKFLADGGCSGGAYDIIICDECHSQDATSILGIGTVLDQAETAGARLTVLATATPPGSITVPHSNIEEVAL

SEQ ID NO: 55 - protein, 88 aa, Homo sapiens
TGNRTITTGAKLTYSTYGKFLADGGCSGGAYDVIICDECHAQDATSILGIGTVLDQAETAGVRLTVLATATPPGSITVPHSNIEEVAL

SEQ ID NO: 56 - protein, 210 aa, Homo sapiens
SVIPTSGDVVVCATDALMTGFTGDFDSVIDCNTCVEQTVDFSLDPTFSIETTTAPQDAVSRSQRRGRTGRGRLGTYRFVTPGERPSGMFDSVVLCECYDAGCAWYELQPAETTVRLRAYLNTPGLPVCQDHLEFWESVFTGLTHIDAHFLSQTKQQGLNFPYLVAYQATVCARAQAPPPSWDEMWKCLVRLKPTLHGPTPLLYRLGAVQN

SEQ ID NO: 57 - protein, 210 aa, Homo sapiens
SVIPTAGDVVVCATDALMTGFTGDFDSVIDCNVAVEQYVDFSLDPTFSIETRTAPQDAVSRSQRRGRTGRGRLGTYRYVGPGERPSGMFDSVVLCECYDAGCAWYELQPAETTVRLRAYLSTPGLPVCQDHLDFWESVFTGLTHIDAHFLSQTKQQGLNFPYLTAYQATVCARAQAPPPSWDEMWKCLVRLKPTLHGPTPLLYRLGPVQN

SEQ ID NO: 58 - protein, 40 aa, Homo sapiens
MACMSADLEVTTSTWVLLGGVLAALAAYCLSTGCVVIVGH

SEQ ID NO: 59 - protein, 40 aa, Homo sapiens
MACMSADLEVTTSTWVLLGGVLAALAAYCLSVGCVVIVGH

SEQ ID NO: 60 - protein, 36 aa, Homo sapiens
FWAKHMWNFISGIQYLAGLSTLPGNPAIASLMAFTA

SEQ ID NO: 61 - protein, 114 aa, Homo sapiens
IGSIGLGKVLVDILAGYGAGVAGALVAFKIMGGELPSTEDMVNLLPAILSPGALVVGVVCAAILRRHVGPGEGAVQWMNRLIAFASRGNHVSPTHYVPESDAAARVTAILSSLT

SEQ ID NO: 62 - protein, 114 aa, Homo sapiens
IGSVGLGKVLVDILAGYGAGVAGALVAFKIMSGEIPSTEDLVNLLPAILSPGALVVGVVCAAILRRHVGPGEGAVQWMNRLIAFASRGNHVSPTHYVPESDAAARVTAILSSLT

SEQ ID NO: 63 - protein, 21 aa, Homo sapiens
CPCQVPAPEFFTEVDGVRLHR

SEQ ID NO: 64 - protein, 20 aa, Homo sapiens
IGSQLPCEPEPDVSVLTSML

SEQ ID NO: 65 - protein, 35 aa, Homo sapiens
TAARRLARGSPPSEASSSASQLSAPSLKATCQTHH

SEQ ID NO: 66 - protein, 35 aa, Homo sapiens
TAARRLARGSPPSEASSSASQLSAPSLKATCQTHR

SEQ ID NO: 67 - protein, 32 aa, Homo sapiens
ESDSESCSSMPPLEGEPGDPDLSDGSWSTVSD

SEQ ID NO: 68 - protein, 32 aa, Homo sapiens
ESDSESCSSMPPLEGEPGDPDLSCDSWSTVSD

SEQ ID NO: 69 - protein, 71 aa, Homo sapiens
QDVVCCSMSYSWTGALITPCAAEEEKLPINPLSNSLLRHHNLVYSTSSRSASQRQKKVTFDRLQVLDDHYK

SEQ ID NO: 70 - protein, 71 aa, Homo sapiens
QSVVCCSMSYSWTGALITPCSAEEEKLPINPLSNSLLRHHNLVYSTSSRSASQRQKKVTFDRLQVLDDHYK

SEQ ID NO: 71 - protein, 30 aa, Homo sapiens
PEKGGRKPARLIVYPDLGVRVCEKMALYDV

SEQ ID NO: 72 - protein, 31 aa, Homo sapiens
WTSKKTPMGFSYDTRCFDSTVTEQDIRVEEE

SEQ ID NO: 73 - protein, 30 aa, Homo sapiens
CGYRRCRASGVLPTSCGNTLTCYIKATAAC

SEQ ID NO: 74 - protein, 30 aa, Homo sapiens
CGYRRCRASGVLTTSCGNTLTCYIKARAAC

SEQ ID NO: 75 - protein, 22 aa, Homo sapiens
ALRAFTEAMTRYSAPPGDAPQP

SEQ ID NO: 76 - protein, 49 aa, Homo sapiens
KGKRVYYLTRDPTTPLARAAWETARHTPVNSWLGNIIMYAPTIWVRMVL

SEQ ID NO: 77 - protein, 49 aa, Homo sapiens
KGKRYYYLTRDPTTPLARAAWETARHTPVNSWLGNIIMYAPTIWVRMVM

SEQ ID NO: 78 - protein, 56 aa, Homo sapiens
YGATYSVEPLDLPAIIERLHGLSAFSLHSYSPGEINRVAGCLRKLGCPPLRAWRHR

SEQ ID NO: 79 - protein, 56 aa, Homo sapiens
YGATYSVTPLDLPAIIERLHGLSAFTLHSYSPVELNRVAGTLRKLGCPPLRAWRHR

SEQ ID NO: 80 - protein, 27 aa, Homo sapiens
VRAKLLSQGGRAAICGKYLFNWAVRTK

SEQ ID NO: 81 - protein, 180 aa, Homo sapiens
TKRNTNRRPQDVKFPGGGQIVGGVYLLPRRGPRLGVRATRKTSERSQPRGRRQPIPKARRPEGRSWAQPGYPWPLYGNEGCGWAGWLLSPRGSRPSWGPNDPRRRSRNLGKVIDTLTCGFADLMGYIPLVGAPVGGVARALAHGVRVLEDGINYATGNLPGCSFSIFLLALLSCLTVPAS

SEQ ID NO: 82 - protein, 180 aa, Homo sapiens
TKRNTNRRPMDVKFPGGGQIVGGVYLLPRRGPRLGVRATRKTSERSQPRGRRQPIPKARRPEGRSWAQPGYPWPLYGNEGCGWAGWLLSPRGSRPSWGPNDPRRRSRNLGKVIDTLTCGFADLMGYIPLVGAPVGGVARALAHGVRALEDGINYATGNLPGCSFSIFLLALLSCLTVPAS

SEQ ID NO: 83 - protein, 27 aa, Homo sapiens
CNCSIYPGHITGHRMAWDMMMNWSPTT

SEQ ID NO: 84 - protein, 22 aa, Homo sapiens
NGSWHINRTALNCNDSLNTGFI

SEQ ID NO: 85 - protein, 44 aa, Homo sapiens
CPTDCFRKHPEATYTKCGSGPWLTPRCLVDYPYRLWHYPCTVNF

SEQ ID NO: 86 - protein, 43 aa, Homo sapiens
LLHSTTEWAILPCSFTTLPALSTGLIHLHQNIVDVQYLYGVGS

SEQ ID NO: 87 - protein, 43 aa, Homo sapiens
LLLSTTEWQILPCSFTTLPALSTGLIHLHQNIVDVQYLYGVGS

SEQ ID NO: 88 - protein, 33 aa, Homo sapiens
KGWRLLAPITAYAQQTRGLLGTIVTSLTGRDKN

SEQ ID NO: 89 - protein, 33 aa, Homo sapiens
MGWRLLAPITAYAQQTRGLLGTIVTSLTGRDKN

SEQ ID NO: 90 - protein, 81 aa, Homo sapiens
PCTCGSSDLYLVTRHADVIPARRRGDSRASLLSPRPISTLKGSSGGPVLCPSGHVVGIFRAAVCTRGVAKALDFIPVESLE

SEQ ID NO: 91 - protein, 81 aa, Homo sapiens
PCTCGSSDLYLVTRHADVIPVRRRGDSRGSLLSPRPISYLKGSSGGPVLCPSGHAVGIFRAAVCTRGVAKAVDFIPVESLE

SEQ ID NO: 92 - protein, 70 aa, Homo sapiens
MRSPVFTDNSTPPAVPQTYQVGHLHAPTGSGKSTKVPAAYAAQGYKVLVLNPSVAATLGFGAYMSKAYGI

SEQ ID NO: 93 - protein, 70 aa, Homo sapiens
MRSPVFTDNSTPPAVPQTYQVAHLHAPTGSGKSTKVPAAYAAQGYKVLVLNPSVAATLGFGAYMSKAYGI

SEQ ID NO: 94 - protein, 75 aa, Homo sapiens
RTGVRTVTTGAPITYSTYGKFLADGGCSGGAYDIIICDECHSTDATTILGIGTVLDQAETAGVRLVVLATATPPG

SEQ ID NO: 95 - protein, 75 aa, Homo sapiens
RSGVRTITTGAPITYSTYGKFLADGGCSGGAYDIIICDECHSTDSTTILGIGTVLDQAETAGVRLVVLATATPPG

SEQ ID NO: 96 - protein, 20 aa, Homo sapiens
IKGGRHLIFCHSKKKCDELA

SEQ ID NO: 97 - protein, 196 aa, Homo sapiens
NAVAYYRGLDVSVIPTSGDVVVCATDALMTGFTGDFDSVIDCNVAVTQTVDFSLDPTFTIETTTVPQDAVSRSQRRGRTGRGRLGIYRYVSPGERPSGMFDSVVLCECYDAGCAWYELTPAETTVRLRAYLNTPGLPVCQDHLEFWEGVFTGLTHIDAHFLSQTKQGGENFPYLVAYQATVCARAKAPPPSWDTMW

SEQ ID NO: 98 - protein, 196 aa, Homo sapiens
NAVAYYRGLDVSVIPTSGDVVVVATDALMTGFTGDFDSVIDCNTCVTQTVDFSLDPTFTIETTTVPQDAVSRSQRRGRTGRGRRGIYRFVTPGERPSGMFDSSVLCECYDAGCAWYELTPAETSVRLRAYLNTPGLPVCQDHLEFWEGVFTGLTHIDAHFLSQTKQAGDNFPYLVAYQATVCARAQAPPPSWDQMW

SEQ ID NO: 99 - protein, 47 aa, Homo sapiens
THPITKYIMACMSADLEVVTSTWVLVGGVLAALAAYCLSVGCVVIVG

SEQ ID NO: 100 - protein, 47 aa, Homo sapiens
THPITKYIMACMSADLEVVTSTWVLVGGVLAALAAYCLSVGSVVIVG

SEQ ID NO: 101 - protein, 42 aa, Homo sapiens
FWAKHMWNFISGIQYLAGLSTLPGNPAVASLMAFTAAVTSPL

SEQ ID NO: 102 - protein, 42 aa, Homo sapiens
FWAKHMWNFISGIQYLAGLSTLPGNPAIASLMAFTAAVTSPL

SEQ ID NO: 103 - protein, 109 aa, Homo sapiens
GAAVGSIGLGKVLVDILAGYGAGVAGALVAFKIMSGEKPSTEDLVNLLPAILSPGALVVGVVCAAILRRHVGPGEGAVQWMNRLIAFASRGNHVSPTHYVPESDAAARV

SEQ ID NO: 104 - protein, 109 aa, Homo sapiens
GAAVGSVGLGKVLVDILAGYGAGVAGALVAFKIMSGEVPSTEDLVNLLPAILSPGALVVGVVCAAILRRHVGPGEGAVQWMNRLIAFASRGNHVSPTHYVPESDAAARV

SEQ ID NO: 105 - protein, 35 aa, Homo sapiens
TAETAARRLARGSPPSLASSSASQLSAPSLKATCT

SEQ ID NO: 106 - protein, 59 aa, Homo sapiens
VCCSMSYSWTGALITPCAAEEEKLPINPLSNSLLRHHNLVYSTTSRSASLRQKKVTFDR

SEQ ID NO: 107 - protein, 59 aa, Homo sapiens
VCCSMSYSWTGALITPCAAEEEKLPINPLSNSLIRHHNMVYSTTSRSASLRQKKVTFDR

SEQ ID NO: 108 - protein, 30 aa, Homo sapiens
PSKGGRKPARLIVYPDLGVRVCEKRALYDV

SEQ ID NO: 109 - protein, 26 aa, Homo sapiens
KKTPMGFSYDTRCFDSTVTERDIRTE

SEQ ID NO: 110 - protein, 29 aa, Homo sapiens
CGYRRCRASGVLTTSMGNTLTCYIKALAA

SEQ ID NO: 111 - protein, 29 aa, Homo sapiens
CGYRRCRASGVLTTSMGNTITCYIKALAA

SEQ ID NO: 112 - protein, 35 aa, Homo sapiens
EAMTRYSAPPGDPPQPEYDLELITSCSSNVSVAHD

SEQ ID NO: 113 - protein, 45 aa, Homo sapiens
TPLARAAWETARHTPVNSWLGNIIMYAPTIWVRMVLMTHFFSILQ

SEQ ID NO: 114 - protein, 31 aa, Homo sapiens
YGATYSVTPLDLPAIIQRLHGLSAFSLHSYS

SEQ ID NO: 115 - protein, 31 aa, Homo sapiens
YGATYSVTPLDLPAIIERLHGLSAFTLHSYS

SEQ ID NO: 116 - protein, 50 aa, Homo sapiens
ELNRVAACLRKLGVPPLRAWRHRARAVRAKLIAQGGRAAICGKYLFNWAV

SEQ ID NO: 117 - protein, 50 aa, Homo sapiens
ELNRVGACLRKLGVPPLRAWRHRARAVRAKLIAQGGKAAICGKYLFNWAV

SEQ ID NO: 118 - protein, 1123 aa, Homo sapiens
MDAMKRGLCCVLLLCGAVFVSPSQEIHARFRRKGGGPGGGKSTNPKPQRKTKRNTNRRPQDVKFPGGGQIVGGVYLLPRRGPRLGVRATRKTSERSQPRGRRQPIPKARRPEGRTWAQPGYPWPLYGNEGCGWAGWLLSPRGSRPSWGPTDPRRRSRNLGKVIDTLTCGFADLMGYIPLVGAPLGGAARALAHGVRVLEDGVNYATGNLPGCSFSIFLLALLSCLTVPASAGGSGDRDRSELSPLLLSTTQWQVLPCSFTTLPALSTGLIHLHQNIVDVQYLYGVGSSVGPPCTCGSSDLYLVTRHADVIPVRRRGDSRGSLLSPRPISYLKGSSGGPLLCPSGHAVGIFRAAVCTRGVAKAVDFIPVESMETTMRSPVFTDNSSPPAVPQTFQVAHLHAPTGSGKSTKVPAAYAAQGYKVLVLNPSVAATLGFGAYMSKAHGVSGTGVRTITTGSPITYSTYGKFLADGGCSGGAYDIIICDECHSTDATSILGIGTVLDQAETAGARLVVLATATPPGSVTVPHPNIEEVGPGNAVAYYRGLDVSVIPTSGDVVVVATDALMTGFTGDFDSVIDCNTCVTQTVDFSLDPTFTIETTTLPQDAVSRTQRRGRTGRGRPGGGSGGGYRFVTPGERPSGMFDSSVLCECYDAGCAWYELTPAETTVRLRAYLNTPGLPVCQDHLEFWEGVFTGLTHIDAHFLSQTKQAGDNFPYLVAYQATVCARAQAPPPSWDQMWKCLIRLKPGGKGPGGKYIMTCMSADLEVVTSTWVLVGGVLAALAAYCLSTGCVVIVGRIVLSGGSGGSIGLGKVLVDILAGYGAGVAGALVAFKIMSGEVPSTEDLVNLLPAILSPGALVVGVVCAAILRRHVGPGEGAVQWMNRLIAFASRGNHVSPTHYVPESDAAARVTQILSGPSLTERLYVGGPLTNSKGQNCGYRRCRASGVLTTSCGNTLTCYLKASAACRAAKLGGPGSLRAFTEAMTRYSAPPGDPPQPEYDLELITSCSSNVSVAHDASGKRVYYLTRDPTTPLARAAWETARHTPVNSWLGNIIMYAPTLWARMILGGSGGEPLDLPQIIQRLHGLSAFSLHSYSPGEINRVAACLRKLGVPPLRAWRHRARSVRA

SEQ ID NO: 119 - protein, 1655 aa, Homo sapiens
MDAMKRGLCCVLLLCGAVFVSPSQEIHARFRRKGGGPGGGKSTNPKPQRKTKRNTNRRPQDVKFPGGGQIVGGVYLLPRRGPRLGVRATRKTSERSQPRGRRQPIPKARRPEGRTWAQPGYPWPLYGNEGCGWAGWLLSPRGSRPSWGPTDPRRRSRNLGKVIDTLTCGFADLMGYIPLVGAPLGGAARALAHGVRVLEDGVNYATGNLPGCSFSIFLLALLSCLTVPASAGGSGYVGDLCGSVFLVSQLFTFSPRPYPGHITGHRMAWDMMMNWSPVCGPVYCFTPSPVVVGTTDRTDVFLLNNTRPPLGNWFGCTWMCPTDCFRKHPEATYSRCGSGPWLTPRCLVDYPYRLWGDRDRSELSPLLLSTTQWQVLPCSFTTLPALSTGLIHLHQNIVDVQYLYGVGSSVARVCACLWMMLLIAQAEAALENLVKGWRLLAPITAYAQQTRGLLGCIITSLTGRDKNQVEGEVQIVSTQSFLATCINGVCWTVYHGAGPCTCGSSDLYLVTRHADVIPVRRRGDSRGSLLSPRPISYLKGSSGGPLLCPSGHAVGIFRAAVCTRGVAKAVDFIPVESMETTMRSPVFTDNSSPPAVPQTFQVAHLHAPTGSGKSTKVPAAYAAQGYKVLVLNPSVAATLGFGAYMSKAHGVSGTGVRTITTGSPITYSTYGKFLADGGCSGGAYDIIICDECHSTDATSILGIGTVLDQAETAGARLVVLATATPPGSVTVPHPNIEEVGPGNAVAYYRGLDVSVIPTSGDVVVVATDALMTGFTGDFDSVIDCNTCVTQTVDFSLDPTFTIETTTLPQDAVSRTQRRGRTGRGRPGGGSGGGYRFVTPGERPSGMFDSSVLCECYDAGCAWYELTPAETTVRLRAYLNTPGLPVCQDHLEFWEGVFTGLTHIDAHFLSQTKQAGDNFPYLVAYQATVCARAQAPPPSWDQMWKCLIRLKPGGKGPGGKYIMTCMSADLEVVTSTWVLVGGVLAALAAYCLSTGCVVIVGRIVLSGGPGFWAKHMWNFISGIQYLAGLSTLPGNPAIASLMAFTASVTSPLTTQPGSIGLGKVLVDILAGYGAGVAGALVAFKIMSGEVPSTEDLVNLLPAILSPGALVVGVVCAAILRRHVGPGEGAVQWMNRLIAFASRGNHVSPTHYVPESDAAARVTQILSSWLRDIWDWICEVLSDFKTWLKCPCQVPSPEFFTELDGVRLHRKKGPGSGPGPRRLARGSPPSLASSSASQLSAPSLKATCTTNHSDAESYSSMPPLEGEPGDPDLSDGSWSTVSSEAGSGSLSNSLLRHHNMVYATTSRSAGPLTPPHSAKSKFGYGAKDVRCHSGSGGGSKPARLIVFPDLGVRVCEKMALYDVVGGPMGFSYDTRCFDSTVTESDIRTEGGSGGGSLTERLYVGGPLTNSKGQNCGYRRCRASGVLTTSCGNTLTCYLKASAACRAAKLGGSGGCTMLVCGDDLVVICESAGTQEDASLRAFTEAMTRYSAPPGDPPQPEYDLELITSCSSNVSVAHDASGKRVYYLTRDPTTPLARAAWETARHTPVNSWLGNIIMYAPTLWARMILGGSGGEPLDLPQIIQRLHGLSAFSLHSYSPGEINRVAACLRKLGVPPLRAWRHRARSVRASGGRAAICGKYLFNWAVRTKLKLTPIPAA

SEQ ID NO: 120 - protein, 1072 aa, Homo sapiens
MDAMKRGLCCVLLLCGAVFVSPSQEIHARFRRKGGGPGGGKSTNPKPQRKTKRNTNRRPQDVKFPGGGQIVGGVYLLPRRGPRLGVRATRKTSERSQPRGRRQPIPKARRPEGRSWAQPGYPWPLYGNEGCGWAGWLLSPRGSRPSWGPTDPRRRSRNLGKVIDTLTCGFADLMGYIPLVGAPLGGAARALAHGVRVLEDGVNYATGNLPGCSFSIFLLALLSCLTVPASGKGGTTELAILPCSFTPLPALSTGLIHLHQNIVDVQYLYGVGSGMMGWRLLAPITAYAQQTRGLLGTIVTSLTGRDKNVVTGEVQVLSTAGSGPCTCGSADLYLVTRDADVIPARRRGDSTASLLSPRPLACLKGSSGGPVMCPSGHVAGIFRAAVCTRGVAKALQFIPVETLRSPVFSDNSSPPAVPQSYQVAHLHAPTGSGKSTKVPAAYAAQGYKVLVLNPSVAATLGFGAYMSKATGNRTITTGAKLTYSTYGKFLADGGCSGGAYDVIICDECHAQDATSILGIGTVLDQAETAGVRLTVLATATPPGSITVPHSNIEEVALSVIPTAGDVVVCATDALMTGFTGDFDSVIDCNVAVEQYVDFSLDPTFSIETRTAPQDAVSRSQRRGRTGRGRLGTYRYVGPGERPSGMFDSVVLCECYDAGCAWYELQPAETTVRLRAYLSTPGLPVCQDHLDFWESVFTGLTHIDAHFLSQTKQQGLNFPYLTAYQATVCARAQAPPPSWDEMWKCLVRLKPTLHGPTPLLYRLGPVQNGGSGKGGIGSVGLGKVLVDILAGYGAGVAGALVAFKIMSGEIPSTEDLVNLLPAILSPGALVVGVVCAAILRRHVGPGEGAVQWMNRLIAFASRGNHVSPTHYVPESDAAARVTAILSSLTSGQSVVCCSMSYSWTGALITPCSAEEEKLPINPLSNSLLRHHNLVYSTSSRSASQRQKKVTFDRLQVLDDHYKKGKRYYYLTRDPTTPLARAAWETARHTPVNSWLGNIIMYAPTIWVRMVMGKGPGSYGATYSVTPLDLPAIIERLHGLSAFTLHSYSPVELNRVAGTLRKLGCPPLRAWRHR

SEQ ID NO: 121 - protein, 1554 aa, Homo sapiens
MDAMKRGLCCVLLLCGAVFVSPSQEIHARFRRKGGGPGGGKSTNPKPQRKTKRNTNRRPQDVKFPGGGQIVGGVYLLPRRGPRLGVRATRKTSERSQPRGRRQPIPKARRPEGRSWAQPGYPWPLYGNEGCGWAGWLLSPRGSRPSWGPTDPRRRSRNLGKVIDTLTCGFADLMGYIPLVGAPLGGAARALAHGVRVLEDGVNYATGNLPGCSFSIFLLALLSCLTVPASGGGSGGGVDLLVGAATMCSALYVGDMCGPHWGVLAGLAYYSMQGNWAKVSVCGPVYCFTPSPVVVGTTDRGPGSGKGPGGRCGSGPWLTPRCLVDYPYRLWHYPCTAACNWTRGERCDIEDRDRSELGGSGTTELAILPCSFTPLPALSTGLIHLHQNIVDVQYLYGVGSGMMGWRLLAPITAYAQQTRGLLGTIVTSLTGRDKNVVTGEVQVLSTAGSGPCTCGSADLYLVTRDADVIPARRRGDSTASLLSPRPLACLKGSSGGPVMCPSGHVAGIFRAAVCTRGVAKALQFIPVETLRSPVFSDNSSPPAVPQSYQVAHLHAPTGSGKSTKVPAAYAAQGYKVLVLNPSVAATLGFGAYMSKATGNRTITTGAKLTYSTYGKFLADGGCSGGAYDVIICDECHAQDATSILGIGTVLDQAETAGVRLTVLATATPPGSITVPHSNIEEVALSVIPTAGDVVVCATDALMTGFTGDFDSVIDCNVAVEQYVDFSLDPTFSIETRTAPQDAVSRSQRRGRTGRGRLGTYRYVGPGERPSGMFDSVVLCECYDAGCAWYELQPAETTVRLRAYLSTPGLPVCQDHLDFWESVFTGLTHIDAHFLSQTKQQGLNFPYLTAYQATVCARAQAPPPSWDEMWKCLVRLKPTLHGPTPLLYRLGPVQNGPPMACMSADLEVTTSTWVLLGGVLAALAAYCLSVGCVVIVGHFWAKHMWNFISGIQYLAGLSTLPGNPAIASLMAFTAGPIGSVGLGKVLVDILAGYGAGVAGALVAFKIMSGEIPSTEDLVNLLPAILSPGALVVGVVCAAILRRHVGPGEGAVQWMNRLIAFASRGNHVSPTHYVPESDAAARVTAILSSLTCPCQVPAPEFFTEVDGVRLHRGGGPPGGGIGSQLPCEPEPDVSVLTSMLPTAARRLARGSPPSEASSSASQLSAPSLKATCQTHRESDSESCSSMPPLEGEPGDPDLSCDSWSTVSDQSVVCCSMSYSWTGALITPCSAEEEKLPINPLSNSLLRHHNLVYSTSSRSASQRQKKVTFDRLQVLDDHYKGPGPEKGGRKPARLIVYPDLGVRVCEKMALYDVPGPGGGWTSKKTPMGFSYDTRCFDSTVTEQDIRVEEEGPCGYRRCRASGVLTTSCGNTLTCYIKARAACGGSGGALRAFTEAMTRYSAPPGDAPQPGGKGKRYYYLTRDPTTPLARAAWETARHTPVNSWLGNIIMYAPTIWVRMVMGKGPGSYGATYSVTPLDLPAIIERLHGLSAFTLHSYSPVELNRVAGTLRKLGCPPLRAWRHRGGPGGPGGVRAKLLSQGGRAAICGKYLFNWAVRTK

SEQ ID NO: 122 - protein, 1115 aa, Homo sapiens
MDAMKRGLCCVLLLCGAVFVSPSQEIHARFRRKGGGPGGGTKRNTNRRPMDVKFPGGGQIVGGVYLLPRRGPRLGVRATRKTSERSQPRGRRQPIPKARRPEGRSWAQPGYPWPLYGNEGCGWAGWLLSPRGSRPSWGPNDPRRRSRNLGKVIDTLTCGFADLMGYIPLVGAPVGGVARALAHGVRALEDGINYATGNLPGCSFSIFLLALLSCLTVPASCPTDCFRKHPEATYTKCGSGPWLTPRCLVDYPYRLWHYPCTVNFGSGLLLSTTEWQILPCSFTTLPALSTGLIHLHQNIVDVQYLYGVGSGPPCTCGSSDLYLVTRHADVIPVRRRGDSRGSLLSPRPISYLKGSSGGPVLCPSGHAVGIFRAAVCTRGVAKAVDFIPVESLEMRSPVFTDNSTPPAVPQTYQVAHLHAPTGSGKSTKVPAAYAAQGYKVLVLNPSVAATLGFGAYMSKAYGIGGSRSGVRTITTGAPITYSTYGKFLADGGCSGGAYDIIICDECHSTDSTTILGIGTVLDQAETAGVRLVVLATATPPGGNAVAYYRGLDVSVIPTSGDVVVVATDALMTGFTGDFDSVIDCNTCVTQTVDFSLDPTFTIETTTVPQDAVSRSQRRGRTGRGRRGIYRFVTPGERPSGMFDSSVLCECYDAGCAWYELTPAETSVRLRAYLNTPGLPVCQDHLEFWEGVFTGLTHIDAHFLSQTKQAGDNFPYLVAYQATVCARAQAPPPSWDQMWTHPITKYIMACMSADLEVVTSTWVLVGGVLAALAAYCLSVGSVVIVGGPGFWAKHMWNFISGIQYLAGLSTLPGNPAIASLMAFTAAVTSPLGAAVGSVGLGKVLVDILAGYGAGVAGALVAFKIMSGEVPSTEDLVNLLPAILSPGALVVGVVCAAILRRHVGPGEGAVQWMNRLIAFASRGNHVSPTHYVPESDAAARVGGGSGGGVCCSMSYSWTGALITPCAAEEEKLPINPLSNSLIRHHNMVYSTTSRSASLRQKKVTFDRGGGKGGGPTPLARAAWETARHTPVNSWLGNIIMYAPTIWVRMVLMTHFFSILQGGGSGGPELNRVGACLRKLGVPPLRAWRHRARAVRAKLIAQGGKAAICGKYLFNWAV

SEQ ID NO: 123 - protein, 1453 aa, Homo sapiens
MDAMKRGLCCVLLLCGAVFVSPSQEIHARFRRKGGGPGGGTKRNTNRRPMDVKFPGGGQIVGGVYLLPRRGPRLGVRATRKTSERSQPRGRRQPIPKARRPEGRSWAQPGYPWPLYGNEGCGWAGWLLSPRGSRPSWGPNDPRRRSRNLGKVIDTLTCGFADLMGYIPLVGAPVGGVARALAHGVRALEDGINYATGNLPGCSFSIFLLALLSCLTVPASPGCNCSIYPGHITGHRMAWDMMMNWSPTTKKNGSWHINRTALNCNDSLNTGFIGPGGSVCGPVYCFTPSPVVVGTTDRGPGCPTDCFRKHPEATYTKCGSGPWLTPRCLVDYPYRLWHYPCTVNFGSGLLLSTTEWQILPCSFTTLPALSTGLIHLHQNIVDVQYLYGVGSMGWRLLAPITAYAQQTRGLLGTIVTSLTGRDKNPCTCGSSDLYLVTRHADVIPVRRRGDSRGSLLSPRPISYLKGSSGGPVLCPSGHAVGIFRAAVCTRGVAKAVDFIPVESLEMRSPVFTDNSTPPAVPQTYQVAHLHAPTGSGKSTKVPAAYAAQGYKVLVLNPSVAATLGFGAYMSKAYGIGGSRSGVRTITTGAPITYSTYGKFLADGGCSGGAYDIIICDECHSTDSTTILGIGTVLDQAETAGVRLVVLATATPPGGKGGKGIKGGRHLIFCHSKKKCDELAGPGNAVAYYRGLDVSVIPTSGDVVVVATDALMTGFTGDFDSVIDCNTCVTQTVDFSLDPTFTIETTTVPQDAVSRSQRRGRTGRGRRGIYRFVTPGERPSGMFDSSVLCECYDAGCAWYELTPAETSVRLRAYLNTPGLPVCQDHLEFWEGVFTGLTHIDAHFLSQTKQAGDNFPYLVAYQATVCARAQAPPPSWDQMWTHPITKYIMACMSADLEVVTSTWVLVGGVLAALAAYCLSVGSVVIVGGPGFWAKHMWNFISGIQYLAGLSTLPGNPAIASLMAFTAAVTSPLGAAVGSVGLGKVLVDILAGYGAGVAGALVAFKIMSGEVPSTEDLVNLLPAILSPGALVVGVVCAAILRRHVGPGEGAVQWMNRLIAFASRGNHVSPTHYVPESDAAARVGPTAETAARRLARGSPPSLASSSASQLSAPSLKATCTVCCSMSYSWTGALITPCAAEEEKLPINPLSNSLIRHHNMVYSTTSRSASLRQKKVTFDRGGSGGPGPSKGGRKPARLIVYPDLGVRVCEKRALYDVPGGPKKTPMGFSYDTRCFDSTVTERDIRTEGGGPGGCGYRRCRASGVLTTSMGNTITCYIKALAAEAMTRYSAPPGDPPQPEYDLELITSCSSNVSVAHDGGSGGTPLARAAWETARHTPVNSWLGNIIMYAPTIWVRMVLMTHFFSILQGGPGYGATYSVTPLDLPAIIERLHGLSAFTLHSYSGGPGGPELNRVGACLRKLGVPPLRAWRHRARAVRAKLIAQGGKAAICGKYLFNWAV

SEQ ID NO: 124 - protein, 1390 aa, Homo sapiens
MDAMKRGLCCVLLLCGAVFVSPSQEIHARFRRKGGGPGGGTKRNTNRRPMDVKFPGGGQIVGGVYLLPRRGPRLGVRATRKTSERSQPRGRRQPIPKARRPEGRSWAQPGYPWPLYGNEGCGWAGWLLSPRGSRPSWGPNDPRRRSRNLGKVIDTLTCGFADLMGYIPLVGAPVGGVARALAHGVRALEDGINYATGNLPGCSFSIFLLALLSCLTVPASCNCSIYPGHITGHRMAWDMMMNWSPTTNGSWHINRTALNCNDSLNTGFISVCGPVYCFTPSPVVVGTTDRCPTDCFRKHPEATYTKCGSGPWLTPRCLVDYPYRLWHYPCTVNFLLLSTTEWQILPCSFTTLPALSTGLIHLHQNIVDVQYLYGVGSMGWRLLAPITAYAQQTRGLLGTIVTSLTGRDKNPCTCGSSDLYLVTRHADVIPVRRRGDSRGSLLSPRPISYLKGSSGGPVLCPSGHAVGIFRAAVCTRGVAKAVDFIPVESLEMRSPVFTDNSTPPAVPQTYQVAHLHAPTGSGKSTKVPAAYAAQGYKVLVLNPSVAATLGFGAYMSKAYGIRSGVRTITTGAPITYSTYGKFLADGGCSGGAYDIIICDECHSTDSTTILGIGTVLDQAETAGVRLVVLATATPPGIKGGRHLIFCHSKKKCDELANAVAYYRGLDVSVIPTSGDVVVVATDALMTGFTGDFDSVIDCNTCVTQTVDFSLDPTFTIETTTVPQDAVSRSQRRGRTGRGRRGIYRFVTPGERPSGMFDSSVLCECYDAGCAWYELTPAETSVRLRAYLNTPGLPVCQDHLEFWEGVFTGLTHIDAHFLSQTKQAGDNFPYLVAYQATVCARAQAPPPSWDQMWTHPITKYIMACMSADLEVVTSTWVLVGGVLAALAAYCLSVGSVVIVGFWAKHMWNFISGIQYLAGLSTLPGNPAIASLMAFTAAVTSPLGAAVGSVGLGKVLVDILAGYGAGVAGALVAFKIMSGEVPSTEDLVNLLPAILSPGALVVGVVCAAILRRHVGPGEGAVQWMNRLIAFASRGNHVSPTHYVPESDAAARVTAETAARRLARGSPPSLASSSASQLSAPSLKATCTVCCSMSYSWTGALITPCAAEEEKLPINPLSNSLIRHHNMVYSTTSRSASLRQKKVTFDRPSKGGRKPARLIVYPDLGVRVCEKRALYDVKKTPMGFSYDTRCFDSTVTERDIRTECGYRRCRASGVLTTSMGNTITCYIKALAAEAMTRYSAPPGDPPQPEYDLELITSCSSNVSVAHDTPLARAAWETARHTPVNSWLGNIIMYAPTIWVRMVLMTHFFSILQYGATYSVTPLDLPAIIERLHGLSAFTLHSYSELNRVGACLRKLGVPPLRAWRHRARAVRAKLIAQGGKAAICGKYLFNWAV

SEQ ID NO: 125 - protein, 1414 aa, Homo sapiens
MTKRNTNRRPMDVKFPGGGQIVGGVYLLPRRGPRLGVRATRKTSERSQPRGRRQPIPKARRPEGRSWAQPGYPWPLYGNEGCGWAGWLLSPRGSRPSWGPNDPRRRSRNLGKVIDTLTCGFADLMGYIPLVGAPVGGVARALAHGVRALEDGINYATGNLPGCSFSIFLLALLSCLTVPASPGCNCSIYPGHITGHRMAWDMMMNWSPTTKKNGSWHINRTALNCNDSLNTGFIGPGGSVCGPVYCFTPSPVVVGTTDRGPGCPTDCFRKHPEATYTKCGSGPWLTPRCLVDYPYRLWHYPCTVNFGSGLLLSTTEWQILPCSFTTLPALSTGLIHLHQNIVDVQYLYGVGSMGWRLLAPITAYAQQTRGLLGTIVTSLTGRDKNPCTCGSSDLYLVTRHADVIPVRRRGDSRGSLLSPRPISYLKGSSGGPVLCPSGHAVGIFRAAVCTRGVAKAVDFIPVESLEMRSPVFTDNSTPPAVPQTYQVAHLHAPTGSGKSTKVPAAYAAQGYKVLVLNPSVAATLGFGAYMSKAYGIGGSRSGVRTITTGAPITYSTYGKFLADGGCSGGAYDIIICDECHSTDSTTILGIGTVLDQAETAGVRLVVLATATPPGGKGGKGIKGGRHLIFCHSKKKCDELAGPGNAVAYYRGLDVSVIPTSGDVVVVATDALMTGFTGDFDSVIDCNTCVTQTVDFSLDPTFTIETTTVPQDAVSRSQRRGRTGRGRRGIYRFVTPGERPSGMFDSSVLCECYDAGCAWYELTPAETSVRLRAYLNTPGLPVCQDHLEFWEGVFTGLTHIDAHFLSQTKQAGDNFPYLVAYQATVCARAQAPPPSWDQMWTHPITKYIMACMSADLEVVTSTWVLVGGVLAALAAYCLSVGSVVIVGGPGFWAKHMWNFISGIQYLAGLSTLPGNPAIASLMAFTAAVTSPLGAAVGSVGLGKVLVDILAGYGAGVAGALVAFKIMSGEVPSTEDLVNLLPAILSPGALVVGVVCAAILRRHVGPGEGAVQWMNRLIAFASRGNHVSPTHYVPESDAAARVGPTAETAARRLARGSPPSLASSSASQLSAPSLKATCTVCCSMSYSWTGALITPCAAEEEKLPINPLSNSLIRHHNMVYSTTSRSASLRQKKVTFDRGGSGGPGPSKGGRKPARLIVYPDLGVRVCEKRALYDVPGGPKKTPMGFSYDTRCFDSTVTERDIRTEGGGPGGCGYRRCRASGVLTTSMGNTITCYIKALAAEAMTRYSAPPGDPPQPEYDLELITSCSSNVSVAHDGGSGGTPLARAAWETARHTPVNSWLGNIIMYAPTIWVRMVLMTHFFSILQGGPGYGATYSVTPLDLPAIIERLHGLSAFTLHSYSGGPGGPELNRVGACLRKLGVPPLRAWRHRARAVRAKLIAQGGKAAICGKYLFNWAV

SEQ ID NO: 126 - protein, 180 aa, Homo sapiens
  VARIANT (65)..(65): X is T or S
  VARIANT (100)..(100): X is T or N
  VARIANT (134)..(134): X is L or V
  VARIANT (137)..(137): X is A or V
  VARIANT (147)..(147): X is V or A
  VARIANT (152)..(152): X is V or I
  VARIANT (154)..(154): X is Y or F
  VARIANT (177)..(177): X is V or H
TKRNTNRRPQDVKFPGGGQIVGGVYLLPRRGPRLGVRATRKTSERSQPRGRRQPIPKARRPEGRXWAQPGYPWPLYGNEGCGWAGWLLSPRGSRPSWGPXDPRRRSRNLGKVIDTLTCGFADLMGYIPLVGAPXGGXARALAHGVRXLEDGXNXATGNLPGCSFSIFLLALLSCLTXPAS

SEQ ID NO: 127 - protein, 20 aa, Homo sapiens
VCGPVYCFTPSPVVVGTTDR

SEQ ID NO: 128 - protein, 21 aa, Homo sapiens
  VARIANT (1)..(1): X is R or K
XCGSGPWLTPRCLVDYPYRLW

SEQ ID NO: 129 - protein, 39 aa, Homo sapiens
  VARIANT (4)..(4): X is W or L
  VARIANT (5)..(5): X is Q or A
  VARIANT (6)..(6): X is V or I
  VARIANT (13)..(13): X is T or P
TTEXXXLPCSFTXLPALSTGLIHLHQNIVDVQYLYGVGS

SEQ ID NO: 130 - protein, 33 aa, Homo sapiens
  VARIANT (1)..(1): X is Q or M or K
  VARIANT (22)..(22): X is C or T
  VARIANT (24)..(24): X is I or V
XGWRLLAPITAYAQQTRGLLGXIXTSLTGRDKN

SEQ ID NO: 131 - protein, 80 aa, Homo sapiens
  VARIANT (21)..(21): X is V or A
  VARIANT (29)..(29): X is G or A
  VARIANT (37)..(37): X is I or L
  VARIANT (38)..(38): X is S or A
  VARIANT (39)..(39): X is Y or T
  VARIANT (48)..(48): X is L or V
  VARIANT (55)..(55): X is A or V
  VARIANT (56)..(56): X is A or V
  VARIANT (72)..(72): X is V or L
  VARIANT (73)..(73): X is D or Q
  VARIANT (79)..(79): X is S or T
PCTCGSSDLYLVTRHADVIPXRRRGDSRXSLLSPRPXXXLKGSSGGPXLCPSGHXXGIFRAAVCTRGVAKAXXFIPVEXL

SEQ ID NO: 132 - protein, 66 aa, Homo sapiens
  VARIANT (4)..(4): X is V or S
  VARIANT (6)..(6): X is T or S
  VARIANT (10)..(10): X is S or T
  VARIANT (17)..(17): X is T or S
  VARIANT (18)..(18): X is F or Y
  VARIANT (21)..(21): X is A or G
RSPXFXDNSXPPAVPQXXQVXHLHAPTGSGKSTKVPAAYAAQGYKVLVLNPSVAATLGFGAYMSKA

SEQ ID NO: 133 - protein, 74 aa, Homo sapiens
  VARIANT (3)..(3): X is V or N
  VARIANT (6)..(6): X is I or V
  VARIANT (11)..(11): X is P or K
  VARIANT (42)..(42): X is T or Q
  VARIANT (46)..(46): X is S or T
  VARIANT (62)..(62): X is A or V
  VARIANT (65)..(65): X is V or T
TGXRTXTTGAXITYSTYGKFLADGGCSGGAYDIIICDECHSXDATXILGIGTVLDQAETAGXRLXVLATATPPG

SEQ ID NO: 134 - protein, 72 aa, Homo sapiens
  VARIANT (12)..(12): X is V or C
  VARIANT (33)..(33): X is T or V
  VARIANT (34)..(34): X is C or A
  VARIANT (36)..(36): X is T or E
  VARIANT (48)..(48): X is T or S
  VARIANT (54)..(54): X is L or A
  VARIANT (62)..(62): X is T or S
SVIPTSGDVVVXATDALMTGFTGDFDSVIDCNXXVXQTVDFSLDPTFXIETTTXPQDAVSRXQRRGRTGRGR

SEQ ID NO: 135 - protein, 110 aa, Homo sapiens
  VARIANT (3)..(3): X is F or Y
  VARIANT (5)..(5): X is T or S
  VARIANT (17)..(17): X is S or V
  VARIANT (33)..(33): X is T or Q
  VARIANT (62)..(62): X is G or S
  VARIANT (81)..(81): X is A or Q or G
  VARIANT (83)..(83): X is E or L
  VARIANT (100)..(100): X is Q or K
  VARIANT (108)..(108): X is Q or E or T
YRXVXPGERPSGMFDSXVLCECYDAGCAWYELXPAETTVRLRAYLNTPGLPVCQDHLEFWEXVFTGLTHIDAHFLSQTKQXGXNFPYLVAYQATVCARAXAPPPSWDXMW

SEQ ID NO: 136 - protein, 39 aa, Homo sapiens
  VARIANT (2)..(2): X is T or A
  VARIANT (11)..(11): X is V or T
  VARIANT (18)..(18): X is V or L
  VARIANT (32)..(32): X is T or V
MXCMSADLEVXTSTWVLXGGVLAALAAYCLSXGCVVIVG

SEQ ID NO: 137 - protein, 36 aa, Homo sapiens
  VARIANT (28)..(28): X is I or V
FWAKHMWNFISGIQYLAGLSTLPGNPAXASLMAFTA

SEQ ID NO: 138 - protein, 105 aa, Homo sapiens
  VARIANT (31)..(31): X is S or G
  VARIANT (34)..(34): X is V or L or K
  VARIANT (40)..(40): X is L or M
GSIGLGKVLVDILAGYGAGVAGALVAFKIMXGEXPSTEDXVNLLPAILSPGALVVGVVCAAILRRHVGPGEGAVQWMNRLIAFASRGNHVSPTHYVPESDAAARV

SEQ ID NO: 139 - protein, 29 aa, Homo sapiens
  VARIANT (11)..(11): X is L or E
  VARIANT (29)..(29): X is T or Q
RRLARGSPPSXASSSASQLSAPSLKATCX

SEQ ID NO: 140 - protein, 26 aa, Homo sapiens
  VARIANT (3)..(3): X is Y or C
  VARIANT (19)..(19): X is S or E
  VARIANT (20)..(20): X is D or F
  VARIANT (21)..(21): X is G or E
  VARIANT (22)..(22): X is S or Q
  VARIANT (23)..(23): X is W or V
  VARIANT (24)..(24): X is S or E
  VARIANT (25)..(25): X is T or S
  VARIANT (26)..(26): X is V or Q
ESXSSMPPLEGEPGDPDLXXXXXXXX

SEQ ID NO: 141 - protein, 20 aa, Homo sapiens
  VARIANT (11)..(11): X is M or L
  VARIANT (14)..(14): X is A or S
  VARIANT (16)..(16): X is T or S
LSNSLLRHHNXVYXTXSRSA

SEQ ID NO: 142 - protein, 24 aa, Homo sapiens
  VARIANT (8)..(8): X is F or Y
  VARIANT (19)..(19): X is M or R
KPARLIVXPDLGVRVCEKXALYDV

SEQ ID NO: 143 - protein, 23 aa, Homo sapiens
  VARIANT (18)..(18): X is S or Q or R
  VARIANT (22)..(22): X is T or V
PMGFSYDTRCFDSTVTEXDIRXE

SEQ ID NO: 144 - protein, 29 aa, Homo sapiens
  VARIANT (13)..(13): X is T or P
  VARIANT (16)..(16): X is C or M
  VARIANT (24)..(24): X is L or I
  VARIANT (27)..(27): X is S or T or L
CGYRRCRASGVLXTSXGNTLTCYXKAXAA

SEQ ID NO: 145 - protein, 16 aa, Homo sapiens
  VARIANT (13)..(13): X is P or A
EAMTRYSAPPGDXPQP

SEQ ID NO: 146 - protein, 36 aa, Homo sapiens
  VARIANT (26)..(26): X is F or Y
  VARIANT (30)..(30): X is L or |
  VARIANT (32)..(32): X is A or V
  VARIANT (35)..(35): X is I or V
TPLARAAWETARHTPVNSWLGNIIMXAPTXWXRMXL

SEQ ID NO: 147 - protein, 24 aa, Homo sapiens
  VARIANT (1)..(1): X is E or T
  VARIANT (7)..(7): X is Q or A
  VARIANT (10)..(10): X is Q or E
XPLDLPXIIXRLHGLSAFSLHSYS

SEQ ID NO: 148 - protein, 23 aa, Homo sapiens
  VARIANT (2)..(2): X is I or L
  VARIANT (7)..(7): X is A or G
  VARIANT (14)..(14): X is V or C
EXNRVAXCLRKLGXPPLRAWRHR

SEQ ID NO: 149 - protein, 16 aa, Homo sapiens
GGRAAICGKYLFNWAV

SEQ ID NO: 150 - protein, 64 aa, Homo sapiens
TKRNTNRRPQDVKFPGGGQIVGGVYLLPRRGPRLGVRATRKTSERSQPRGRRQPIPKARRPEGR

SEQ ID NO: 151 - protein, 34 aa, Homo sapiens
WAQPGYPWPLYGNEGCGWAGWLLSPRGSRPSWGP

SEQ ID NO: 152 - protein, 33 aa, Homo sapiens
DPRRRSRNLGKVIDTLTCGFADLMGYIPLVGAP

SEQ ID NO: 153 - protein, 9 aa, Homo sapiens
ARALAHGVR

SEQ ID NO: 154 - protein, 22 aa, Homo sapiens
ATGNLPGCSFSIFLLALLSCLT

SEQ ID NO: 155 - protein, 20 aa, Homo sapiens
VCGPVYCFTPSPVVVGTTDR

SEQ ID NO: 156 - protein, 20 aa, Homo sapiens
CGSGPWLTPRCLVDYPYRLW

SEQ ID NO: 157 - protein, 26 aa, Homo sapiens
LPALSTGLIHLHQNIVDVQYLYGVGS

SEQ ID NO: 158 - protein, 20 aa, Homo sapiens
GWRLLAPITAYAQQTRGLLG

SEQ ID NO: 159 - protein, 9 aa, Homo sapiens
TSLTGRDKN

SEQ ID NO: 160 - protein, 20 aa, Homo sapiens
PCTCGSSDLYLVTRHADVIP

SEQ ID NO: 161 - protein, 8 aa, Homo sapiens
LKGSSGGP

SEQ ID NO: 162 - protein, 15 aa, Homo sapiens
GIFRAAVCTRGVAKA

SEQ ID NO: 163 - protein, 45 aa, Homo sapiens
HLHAPTGSGKSTKVPAAYAAQGYKVLVLNPSVAATLGFGAYMSKA

SEQ ID NO: 164 - protein, 30 aa, Homo sapiens
ITYSTYGKFLADGGCSGGAYDIIICDECHS

SEQ ID NO: 165 - protein, 15 aa, Homo sapiens
ILGIGTVLDQAETAG

SEQ ID NO: 166 - protein, 9 aa, Homo sapiens
VLATATPPG

SEQ ID NO: 167 - protein, 11 aa, Homo sapiens
SVIPTSGDVVV

SEQ ID NO: 168 - protein, 20 aa, Homo sapiens
ATDALMTGFTGDFDSVIDCN

SEQ ID NO: 169 - protein, 11 aa, Homo sapiens
QTVDFSLDPTF

SEQ ID NO: 170 - protein, 10 aa, Homo sapiens
QRRGRTGRGR

SEQ ID NO: 171 - protein, 11 aa, Homo sapiens
PGERPSGMFDS

SEQ ID NO: 172 - protein, 15 aa, Homo sapiens
VLCECYDAGCAWYEL

SEQ ID NO: 173 - protein, 28 aa, Homo sapiens
PAETTVRLRAYLNTPGLPVCQDHLEFWE

SEQ ID NO: 174 - protein, 18 aa, Homo sapiens
VFTGLTHIDAHFLSQTKQ

SEQ ID NO: 175 - protein, 16 aa, Homo sapiens
NFPYLVAYQATVCARA

SEQ ID NO: 176 - protein, 8 aa, Homo sapiens
CMSADLEV

SEQ ID NO: 177 - protein, 13 aa, Homo sapiens
GGVLAALAAYCLS

SEQ ID NO: 178 - protein, 27 aa, Homo sapiens
FWAKHMWNFISGIQYLAGLSTLPGNPA

SEQ ID NO: 179 - protein, 8 aa, Homo sapiens
ASLMAFTA

SEQ ID NO: 180 - protein, 30 aa, Homo sapiens
GSIGLGKVLVDILAGYGAGVAGALVAFKIM

SEQ ID NO: 181 - protein, 65 aa, Homo sapiens
VNLLPAILSPGALVVGVVCAAILRRHVGPGEGAVQWMNRLIAFASRGNHVSPTHYVPESDAAARV

SEQ ID NO: 182 - protein, 10 aa, Homo sapiens
RRLARGSPPS

SEQ ID NO: 183 - protein, 17 aa, Homo sapiens
ASSSASQLSAPSLKATC

SEQ ID NO: 184 - protein, 15 aa, Homo sapiens
SSMPPLEGEPGDPDL

SEQ ID NO: 185 - protein, 9 aa, Homo sapiens
LSNSLLRHH

SEQ ID NO: 186 - protein, 10 aa, Homo sapiens
PDLGVRVCEK

SEQ ID NO: 187 - protein, 17 aa, Homo sapiens
PMGFSYDTRCFDSTVTE

SEQ ID NO: 188 - protein, 12 aa, Homo sapiens
CGYRRCRASGVL

SEQ ID NO: 189 - protein, 12 aa, Homo sapiens
EAMTRYSAPPGD

SEQ ID NO: 190 - protein, 25 aa, Homo sapiens
TPLARAAWETARHTPVNSWLGNIIM

SEQ ID NO: 191 - protein, 14 aa, Homo sapiens
RLHGLSAFSLHSYS

SEQ ID NO: 192 - protein, 9 aa, Homo sapiens
PPLRAWRHR

SEQ ID NO: 193 - protein, 16 aa, Homo sapiens
GGRAAICGKYLFNWAV

SEQ ID NO: 194 - protein, 32 aa, Homo sapiens
MDAMKRGLCCVLLLCGAVFVSPSQEIHARFRR

SEQ ID NO: 195 - protein, 27 aa, Homo sapiens
SLLWGGVTVLAAMLIAGQVASSVVFLV